European Patent Application EP 4 506 366 A1, published February 12, 2025. Title: ANTIGEN-BINDING PROTEIN TARGETING PD-L1 AND CD40, PREPARATION THEREFOR, AND USE THEREOF. Applicant: HARBOUR BIOMED (SHANGHAI) CO., LTD. Application EP. The sequence listing filed with the application follows.

SEQUENCE LISTING (106 sequences)

SEQ ID NO: 1 - protein, 25 aa, synthetic construct [sequence omitted]

SEQ ID NO: 2 - protein, 25 aa, synthetic construct
QVQLVESGGGVVQPGMSLRLSCAAS

SEQ ID NO: 3 - protein, 25 aa, synthetic construct [sequence omitted]

SEQ ID NO: 4 - protein, 7 aa, synthetic construct
GFTFSDS

SEQ ID NO: 5 - protein, 7 aa, synthetic construct
GFNFSNY

SEQ ID NO: 6 - protein, 7 aa, synthetic construct
GYTFTGY

SEQ ID NO: 7 - protein, 7 aa, synthetic construct
GFTFSSY

SEQ ID NO: 8 - protein, 7 aa, synthetic construct
GYTFAGY

SEQ ID NO: 9 - protein, 7 aa, synthetic construct
GFDFSSY

SEQ ID NO: 10 - protein, 19 aa, synthetic construct
WIHWVRQAPGKGLEWVAWI

SEQ ID NO: 11 - protein, 19 aa, synthetic construct
GMYWVRQAPGKGQEWVAII

SEQ ID NO: 12 - protein, 19 aa, synthetic construct
YMHWVRQAPGQGLEWMGWI

SEQ ID NO: 13 - protein, 19 aa, synthetic construct
YMYWVRQAPGQGLEWMGWI

SEQ ID NO: 14 - protein, 19 aa, synthetic construct
GMYWVRQAPGKGQEWVASI

SEQ ID NO: 15 - protein, 6 aa, synthetic construct
SPYGGS

SEQ ID NO: 16 - protein, 6 aa, synthetic construct
WYDGTK

SEQ ID NO: 17 - protein, 6 aa, synthetic construct
NPDSGG

SEQ ID NO: 18 - protein, 6 aa, synthetic construct
NPDSGA

SEQ ID NO: 19 - protein, 6 aa, synthetic construct
RYTGTE

SEQ ID NO: 20 - protein, 41 aa, synthetic construct
TYYADSVKGRFTISADTSKNTAYLQMNSLRAEDTAVYYCAR

SEQ ID NO: 21 - protein, 41 aa, synthetic construct
KHYADSVKGRFTISRDNSKNTLYLEMNSLRVEDTAVYYCAK

SEQ ID NO: 22 - protein, 41 aa, synthetic construct
TNYAQKFQGRVTMTRDTSISTAYMELNRLRSDDTAVYYCAR

SEQ ID NO: 23 - protein, 41 aa, synthetic construct
PTYAQKFQGRVTMTRDTSISTAYMELSRLRSDDTAVYYCAR

SEQ ID NO: 24 - protein, 9 aa, synthetic construct
RHWPGGFDY

SEQ ID NO: 25 - protein, 14 aa, synthetic construct
NRAIFGVVPDASDI

SEQ ID NO: 26 - protein, 17 aa, synthetic construct
DQPLGYCTNGVCSYFDY

SEQ ID NO: 27 - protein, 16 aa, synthetic construct
EKIYYGSGNYYPSFDY

SEQ ID NO: 28 - protein, 14 aa, synthetic construct
NRALFGVIPDDSDI

SEQ ID NO: 29 - protein, 14 aa, synthetic construct
NRAIFGVIPDDSDI

SEQ ID NO: 30 - protein, 14 aa, synthetic construct
NRALFGVIPDASDI

SEQ ID NO: 31 - protein, 11 aa, synthetic construct
WGQGTLVTVSS

SEQ ID NO: 32 - protein, 11 aa, synthetic construct
RGQGTMVTVSS

SEQ ID NO: 33 - protein, 23 aa, synthetic construct
DIQMTQSPSSLSASVGDRVTITC

SEQ ID NO: 34 - protein, 23 aa, synthetic construct
DIQMTQSPSSVSASVGDRVTITC

SEQ ID NO: 35 - protein, 23 aa, synthetic construct
DIQLTQSPSFLSASVGDRVTITC

SEQ ID NO: 36 - protein, 11 aa, synthetic construct
RASQDVSTAVA

SEQ ID NO: 37 - protein, 11 aa, synthetic construct
RASQGIYSWLA

SEQ ID NO: 38 - protein, 11 aa, synthetic construct
RASQGISSYLA

SEQ ID NO: 39 - protein, 15 aa, synthetic construct
WYQQKPGKAPKLLIY

SEQ ID NO: 40 - protein, 15 aa, synthetic construct
WYQQKPGKAPNLLIY

SEQ ID NO: 41 - protein, 7 aa, synthetic construct
SASFLYS

SEQ ID NO: 42 - protein, 7 aa, synthetic construct
TASTLQS

SEQ ID NO: 43 - protein, 7 aa, synthetic construct
AASTLQS

SEQ ID NO: 44 - protein, 32 aa, synthetic construct
GVPSRFSGSGSGTDFTLTISSLQPEDFATYYC

SEQ ID NO: 45 - protein, 32 aa, synthetic construct
GVPSRFSGSGSGTEFTLTISSLQPEDFATYYC

SEQ ID NO: 46 - protein, 9 aa, synthetic construct
QQYLYHPAT

SEQ ID NO: 47 - protein, 9 aa, synthetic construct
QQANIFPLT

SEQ ID NO: 48 - protein, 9 aa, synthetic construct
QQLNSYPWT

SEQ ID NO: 49 - protein, 9 aa, synthetic construct
QQLASYPWT

SEQ ID NO: 50 - protein, 9 aa, synthetic construct
QQLFSYPWT

SEQ ID NO: 51 - protein, 9 aa, synthetic construct
QQLYSYPWT

SEQ ID NO: 52 - protein, 9 aa, synthetic construct
QQLVSYPWT

SEQ ID NO: 53 - protein, 9 aa, synthetic construct
QQLNNYPWT

SEQ ID NO: 54 - protein, 10 aa, synthetic construct
FGQGTKVEIK

SEQ ID NO: 55 - protein, 10 aa, synthetic construct
FGGGTKVEIK

SEQ ID NO: 56 - protein, 118 aa, synthetic construct [sequence omitted]

SEQ ID NO: 57 - protein, 123 aa, synthetic construct
QVQLVESGGGVVQPGMSLRLSCAASGFNFSNYGMYWVRQAPGKGQEWVAIIWYDGTKKHYADSVKGRFTISRDNSKNTLYLEMNSLRVEDTAVYYCAKNRAIFGVVPDASDIRGQGTMVTVSS

SEQ ID NO: 58 - protein, 126 aa, synthetic construct
QVQLVQSGAEVKKPGASVKVSCKASGYTFTGYYMHWVRQAPGQGLEWMGWINPDSGGTNYAQKFQGRVTMTRDTSISTAYMELNRLRSDDTAVYYCARDQPLGYCTNGVCSYFDYWGQGTLVTVSS

SEQ ID NO: 59 - protein, 123 aa, synthetic construct
QVQLVESGGGVVQPGMSLRLSCAASGFTFSSYGMYWVRQAPGKGQEWVAIIWYDGTKKHYADSVKGRFTISRDNSKNTLYLEMNSLRVEDTAVYYCAKNRAIFGVVPDASDIRGQGTMVTVSS

SEQ ID NO: 60 - protein, 125 aa, synthetic construct
QVQLVQSGAEVKKPGASVKVSCKASGYTFAGYYMYWVRQAPGQGLEWMGWINPDSGAPTYAQKFQGRVTMTRDTSISTAYMELSRLRSDDTAVYYCAREKIYYGSGNYYPSFDYWGQGTLVTVSS

SEQ ID NO: 61 - protein, 123 aa, synthetic construct
QVQLVESGGGVVQPGMSLRLSCAASGFTFSSYGMYWVRQAPGKGQEWVASIRYTGTEKHYADSVKGRFTISRDNSKNTLYLEMNSLRVEDTAVYYCAKNRALFGVIPDDSDIRGQGTMVTVSS

SEQ ID NO: 62 - protein, 123 aa, synthetic construct
QVQLVESGGGVVQPGMSLRLSCAASGFDFSSYGMYWVRQAPGKGQEWVASIRYTGTEKHYADSVKGRFTISRDNSKNTLYLEMNSLRVEDTAVYYCAKNRAIFGVVPDASDIRGQGTMVTVSS

SEQ ID NO: 63 - protein, 123 aa, synthetic construct
QVQLVESGGGVVQPGMSLRLSCAASGFDFSSYGMYWVRQAPGKGQEWVASIRYTGTEKHYADSVKGRFTISRDNSKNTLYLEMNSLRVEDTAVYYCAKNRAIFGVIPDDSDIRGQGTMVTVSS

SEQ ID NO: 64 - protein, 123 aa, synthetic construct
QVQLVESGGGVVQPGMSLRLSCAASGFDFSSYGMYWVRQAPGKGQEWVASIRYTGTEKHYADSVKGRFTISRDNSKNTLYLEMNSLRVEDTAVYYCAKNRALFGVIPDASDIRGQGTMVTVSS

SEQ ID NO: 65 - protein, 123 aa, synthetic construct
QVQLVESGGGVVQPGMSLRLSCAASGFDFSSYGMYWVRQAPGKGQEWVASIRYTGTEKHYADSVKGRFTISRDNSKNTLYLEMNSLRVEDTAVYYCAKNRALFGVIPDDSDIRGQGTMVTVSS

SEQ ID NO: 66 - protein, 107 aa, synthetic construct [sequence omitted]

SEQ ID NO: 67 - protein, 107 aa, synthetic construct
DIQMTQSPSSVSASVGDRVTITCRASQGIYSWLAWYQQKPGKAPNLLIYTASTLQSGVPSRFSGSGSGTDFTLTISSLQPEDFATYYCQQANIFPLTFGGGTKVEIK

SEQ ID NO: 68 - protein, 107 aa, synthetic construct
DIQLTQSPSFLSASVGDRVTITCRASQGISSYLAWYQQKPGKAPKLLIYAASTLQSGVPSRFSGSGSGTEFTLTISSLQPEDFATYYCQQLNSYPWTFGQGTKVEIK

SEQ ID NO: 69 - protein, 107 aa, synthetic construct
DIQLTQSPSFLSASVGDRVTITCRASQGISSYLAWYQQKPGKAPKLLIYAASTLQSGVPSRFSGSGSGTEFTLTISSLQPEDFATYYCQQLASYPWTFGQGTKVEIK

SEQ ID NO: 70 - protein, 107 aa, synthetic construct
DIQLTQSPSFLSASVGDRVTITCRASQGISSYLAWYQQKPGKAPKLLIYAASTLQSGVPSRFSGSGSGTEFTLTISSLQPEDFATYYCQQLFSYPWTFGQGTKVEIK

SEQ ID NO: 71 - protein, 107 aa, synthetic construct
DIQLTQSPSFLSASVGDRVTITCRASQGISSYLAWYQQKPGKAPKLLIYAASTLQSGVPSRFSGSGSGTEFTLTISSLQPEDFATYYCQQLYSYPWTFGQGTKVEIK

SEQ ID NO: 72 - protein, 107 aa, synthetic construct
DIQLTQSPSFLSASVGDRVTITCRASQGISSYLAWYQQKPGKAPKLLIYAASTLQSGVPSRFSGSGSGTEFTLTISSLQPEDFATYYCQQLVSYPWTFGQGTKVEIK

SEQ ID NO: 73 - protein, 107 aa, synthetic construct
DIQLTQSPSFLSASVGDRVTITCRASQGISSYLAWYQQKPGKAPKLLIYAASTLQSGVPSRFSGSGSGTEFTLTISSLQPEDFATYYCQQLNNYPWTFGQGTKVEIK

SEQ ID NO: 74 - protein, 448 aa, synthetic construct
EVQLVESGGGLVQPGGSLRLSCAASGFTFSDSWIHWVRQAPGKGLEWVAWISPYGGSTYYADSVKGRFTISADTSKNTAYLQMNSLRAEDTAVYYCARRHWPGGFDYWGQGTLVTVSSASTKGPSVFPLAPSSKSTSGGTAALGCLVKDYFPEPVTVSWNSGALTSGVHTFPAVLQSSGLYSLSSVVTVPSSSLGTQTYICNVNHKPSNTKVDKKVEPKSCDKTHTCPPCPAPELLGGPSVFLFPPKPKDTLMISRTPEVTCVVVDVSHEDPEVKFNWYVDGVEVHNAKTKPREEQYASTYRVVSVLTVLHQDWLNGKEYKCKVSNKALPAPIEKTISKAKGQPREPQVYTLPPSREEMTKNQVSLTCLVKGFYPSDIAVEWESNGQPENNYKTTPPVLDSDGSFFLYSKLTVDKSRWQQGNVFSCSVMHEALHNHYTQKSLSLSPGK

SEQ ID NO: 75 - protein, 355 aa, synthetic construct
QVQLVESGGGVVQPGMSLRLSCAASGFNFSNYGMYWVRQAPGKGQEWVAIIWYDGTKKHYADSVKGRFTISRDNSKNTLYLEMNSLRVEDTAVYYCAKNRAIFGVVPDASDIRGQGTMVTVSSEPKSCDKTHTCPPCPAPELLGGPSVFLFPPKPKDTLMISRTPEVTCVVVDVSHEDPEVKFNWYVDGVEVHNAKTKPREEQYNSTYRVVSVLTVLHQDWLNGKEYKCKVSNKALPAPIEKTISKAKGQPREPQVYTLPPSREEMTKNQVSLTCLVKGFYPSDIAVEWESNGQPENNYKTTPPVLDSDGSFFLYSKLTVDKSRWQQGNVFSCSVMHEALHNHYTQKSLSLSPGK

SEQ ID NO: 76 - protein, 452 aa, synthetic construct
QVQLVQSGAEVKKPGASVKVSCKASGYTFTGYYMHWVRQAPGQGLEWMGWINPDSGGTNYAQKFQGRVTMTRDTSISTAYMELNRLRSDDTAVYYCARDQPLGYCTNGVCSYFDYWGQGTLVTVSSASTKGPSVFPLAPCSRSTSESTAALGCLVKDYFPEPVTVSWNSGALTSGVHTFPAVLQSSGLYSLSSVVTVPSSNFGTQTYTCNVDHKPSNTKVDKTVERKCCVECPPCPAPPVAGPSVFLFPPKPKDTLMISRTPEVTCVVVDVSHEDPEVQFNWYVDGVEVHNAKTKPREEQFNSTFRVVSVLTVVHQDWLNGKEYKCKVSNKGLPAPIEKTISKTKGQPREPQVYTLPPSREEMTKNQVSLTCLVKGFYPSDIAVEWESNGQPENNYKTTPPMLDSDGSFFLYSKLTVDKSRWQQGNVFSCSVMHEALHNHYTQKSLSLSPGK

SEQ ID NO: 77 - protein, 355 aa, synthetic construct
QVQLVESGGGVVQPGMSLRLSCAASGFTFSSYGMYWVRQAPGKGQEWVAIIWYDGTKKHYADSVKGRFTISRDNSKNTLYLEMNSLRVEDTAVYYCAKNRAIFGVVPDASDIRGQGTMVTVSSEPKSCDKTHTCPPCPAPELLGGPSVFLFPPKPKDTLMISRTPEVTCVVVDVSHEDPEVKFNWYVDGVEVHNAKTKPREEQYNSTYRVVSVLTVLHQDWLNGKEYKCKVSNKALPAPIEKTISKAKGQPREPQVYTLPPSREEMTKNQVSLTCLVKGFYPSDIAVEWESNGQPENNYKTTPPVLDSDGSFFLYSKLTVDKSRWQQGNVFSCSVMHEALHNHYTQKSLSLSPGK

SEQ ID NO: 78 - protein, 451 aa, synthetic construct
QVQLVQSGAEVKKPGASVKVSCKASGYTFAGYYMYWVRQAPGQGLEWMGWINPDSGAPTYAQKFQGRVTMTRDTSISTAYMELSRLRSDDTAVYYCAREKIYYGSGNYYPSFDYWGQGTLVTVSSASTKGPSVFPLAPCSRSTSESTAALGCLVKDYFPEPVTVSWNSGALTSGVHTFPAVLQSSGLYSLSSVVTVPSSNFGTQTYTCNVDHKPSNTKVDKTVERKCCVECPPCPAPPVAGPSVFLFPPKPKDTLMISRTPEVTCVVVDVSHEDPEVQFNWYVDGVEVHNAKTKPREEQFNSTFRVVSVLTVVHQDWLNGKEYKCKVSNKGLPAPIEKTISKTKGQPREPQVYTLPPSREEMTKNQVSLTCLVKGFYPSDIAVEWESNGQPENNYKTTPPMLDSDGSFFLYSKLTVDKSRWQQGNVFSCSVMHEALHNHYTQKSLSLSPGK

SEQ ID NO: 79 - protein, 355 aa, synthetic construct
QVQLVESGGGVVQPGMSLRLSCAASGFTFSSYGMYWVRQAPGKGQEWVASIRYTGTEKHYADSVKGRFTISRDNSKNTLYLEMNSLRVEDTAVYYCAKNRALFGVIPDDSDIRGQGTMVTVSSEPKSCDKTHTCPPCPAPELLGGPSVFLFPPKPKDTLMISRTPEVTCVVVDVSHEDPEVKFNWYVDGVEVHNAKTKPREEQYNSTYRVVSVLTVLHQDWLNGKEYKCKVSNKALPAPIEKTISKAKGQPREPQVYTLPPSREEMTKNQVSLTCLVKGFYPSDIAVEWESNGQPENNYKTTPPVLDSDGSFFLYSKLTVDKSRWQQGNVFSCSVMHEALHNHYTQKSLSLSPGK

SEQ ID NO: 80 - protein, 355 aa, synthetic construct
QVQLVESGGGVVQPGMSLRLSCAASGFDFSSYGMYWVRQAPGKGQEWVASIRYTGTEKHYADSVKGRFTISRDNSKNTLYLEMNSLRVEDTAVYYCAKNRAIFGVVPDASDIRGQGTMVTVSSEPKSCDKTHTCPPCPAPELLGGPSVFLFPPKPKDTLMISRTPEVTCVVVDVSHEDPEVKFNWYVDGVEVHNAKTKPREEQYNSTYRVVSVLTVLHQDWLNGKEYKCKVSNKALPAPIEKTISKAKGQPREPQVYTLPPSREEMTKNQVSLTCLVKGFYPSDIAVEWESNGQPENNYKTTPPVLDSDGSFFLYSKLTVDKSRWQQGNVFSCSVMHEALHNHYTQKSLSLSPGK

SEQ ID NO: 81 - protein, 355 aa, synthetic construct
QVQLVESGGGVVQPGMSLRLSCAASGFDFSSYGMYWVRQAPGKGQEWVASIRYTGTEKHYADSVKGRFTISRDNSKNTLYLEMNSLRVEDTAVYYCAKNRAIFGVIPDDSDIRGQGTMVTVSSEPKSCDKTHTCPPCPAPELLGGPSVFLFPPKPKDTLMISRTPEVTCVVVDVSHEDPEVKFNWYVDGVEVHNAKTKPREEQYNSTYRVVSVLTVLHQDWLNGKEYKCKVSNKALPAPIEKTISKAKGQPREPQVYTLPPSREEMTKNQVSLTCLVKGFYPSDIAVEWESNGQPENNYKTTPPVLDSDGSFFLYSKLTVDKSRWQQGNVFSCSVMHEALHNHYTQKSLSLSPGK

SEQ ID NO: 82 - protein, 355 aa, synthetic construct
QVQLVESGGGVVQPGMSLRLSCAASGFDFSSYGMYWVRQAPGKGQEWVASIRYTGTEKHYADSVKGRFTISRDNSKNTLYLEMNSLRVEDTAVYYCAKNRALFGVIPDASDIRGQGTMVTVSSEPKSCDKTHTCPPCPAPELLGGPSVFLFPPKPKDTLMISRTPEVTCVVVDVSHEDPEVKFNWYVDGVEVHNAKTKPREEQYNSTYRVVSVLTVLHQDWLNGKEYKCKVSNKALPAPIEKTISKAKGQPREPQVYTLPPSREEMTKNQVSLTCLVKGFYPSDIAVEWESNGQPENNYKTTPPVLDSDGSFFLYSKLTVDKSRWQQGNVFSCSVMHEALHNHYTQKSLSLSPGK

SEQ ID NO: 83 - protein, 355 aa, synthetic construct
QVQLVESGGGVVQPGMSLRLSCAASGFDFSSYGMYWVRQAPGKGQEWVASIRYTGTEKHYADSVKGRFTISRDNSKNTLYLEMNSLRVEDTAVYYCAKNRALFGVIPDDSDIRGQGTMVTVSSEPKSCDKTHTCPPCPAPELLGGPSVFLFPPKPKDTLMISRTPEVTCVVVDVSHEDPEVKFNWYVDGVEVHNAKTKPREEQYNSTYRVVSVLTVLHQDWLNGKEYKCKVSNKALPAPIEKTISKAKGQPREPQVYTLPPSREEMTKNQVSLTCLVKGFYPSDIAVEWESNGQPENNYKTTPPVLDSDGSFFLYSKLTVDKSRWQQGNVFSCSVMHEALHNHYTQKSLSLSPGK

SEQ ID NO: 84 - protein, 455 aa, synthetic construct
QVQLVQSGAEVKKPGASVKVSCKASGYTFAGYYMYWVRQAPGQGLEWMGWINPDSGAPTYAQKFQGRVTMTRDTSISTAYMELSRLRSDDTAVYYCAREKIYYGSGNYYPSFDYWGQGTLVTVSSASTKGPSVFPLAPSSKSTSGGTAALGCLVKDYFPEPVTVSWNSGALTSGVHTFPAVLQSSGLYSLSSVVTVPSSSLGTQTYICNVNHKPSNTKVDKKVEPKSCDKTHTCPPCPAPEAAGAPSVFLFPPKPKDTLMISRTPEVTCVVVDVSHEDPEVKFNWYVDGVEVHNAKTKPREEQYNSTYRVVSVLTVLHQDWLNGKEYKCKVSNKALPAPIEKTISKAKGQPREPQVYTLPPSREEMTKNQVSLTCLVKGFYPSDIAVEWESNGQPENNYKTTPPVLDSDGSFFLYSKLTVDKSRWQQGNVFSCSVMHEALHNHYTQKSLSLSPGK

SEQ ID NO: 85 - protein, 214 aa, synthetic construct
DIQMTQSPSSLSASVGDRVTITCRASQDVSTAVAWYQQKPGKAPKLLIYSASFLYSGVPSRFSGSGSGTDFTLTISSLQPEDFATYYCQQYLYHPATFGQGTKVEIKRTVAAPSVFIFPPSDEQLKSGTASVVCLLNNFYPREAKVQWKVDNALQSGNSQESVTEQDSKDSTYSLSSTLTLSKADYEKHKVYACEVTHQGLSSPVTKSFNRGEC

SEQ ID NO: 86 - protein, 214 aa, synthetic construct
DIQMTQSPSSVSASVGDRVTITCRASQGIYSWLAWYQQKPGKAPNLLIYTASTLQSGVPSRFSGSGSGTDFTLTISSLQPEDFATYYCQQANIFPLTFGGGTKVEIKRTVAAPSVFIFPPSDEQLKSGTASVVCLLNNFYPREAKVQWKVDNALQSGNSQESVTEQDSKDSTYSLSSTLTLSKADYEKHKVYACEVTHQGLSSPVTKSFNRGEC

SEQ ID NO: 87 - protein, 214 aa, synthetic construct
DIQLTQSPSFLSASVGDRVTITCRASQGISSYLAWYQQKPGKAPKLLIYAASTLQSGVPSRFSGSGSGTEFTLTISSLQPEDFATYYCQQLNSYPWTFGQGTKVEIKRTVAAPSVFIFPPSDEQLKSGTASVVCLLNNFYPREAKVQWKVDNALQSGNSQESVTEQDSKDSTYSLSSTLTLSKADYEKHKVYACEVTHQGLSSPVTKSFNRGEC

SEQ ID NO: 88 - protein, 214 aa, synthetic construct
DIQLTQSPSFLSASVGDRVTITCRASQGISSYLAWYQQKPGKAPKLLIYAASTLQSGVPSRFSGSGSGTEFTLTISSLQPEDFATYYCQQLASYPWTFGQGTKVEIKRTVAAPSVFIFPPSDEQLKSGTASVVCLLNNFYPREAKVQWKVDNALQSGNSQESVTEQDSKDSTYSLSSTLTLSKADYEKHKVYACEVTHQGLSSPVTKSFNRGEC

SEQ ID NO: 89 - protein, 214 aa, synthetic construct
DIQLTQSPSFLSASVGDRVTITCRASQGISSYLAWYQQKPGKAPKLLIYAASTLQSGVPSRFSGSGSGTEFTLTISSLQPEDFATYYCQQLFSYPWTFGQGTKVEIKRTVAAPSVFIFPPSDEQLKSGTASVVCLLNNFYPREAKVQWKVDNALQSGNSQESVTEQDSKDSTYSLSSTLTLSKADYEKHKVYACEVTHQGLSSPVTKSFNRGEC

SEQ ID NO: 90 - protein, 214 aa, synthetic construct
DIQLTQSPSFLSASVGDRVTITCRASQGISSYLAWYQQKPGKAPKLLIYAASTLQSGVPSRFSGSGSGTEFTLTISSLQPEDFATYYCQQLYSYPWTFGQGTKVEIKRTVAAPSVFIFPPSDEQLKSGTASVVCLLNNFYPREAKVQWKVDNALQSGNSQESVTEQDSKDSTYSLSSTLTLSKADYEKHKVYACEVTHQGLSSPVTKSFNRGEC

SEQ ID NO: 91 - protein, 214 aa, synthetic construct
DIQLTQSPSFLSASVGDRVTITCRASQGISSYLAWYQQKPGKAPKLLIYAASTLQSGVPSRFSGSGSGTEFTLTISSLQPEDFATYYCQQLVSYPWTFGQGTKVEIKRTVAAPSVFIFPPSDEQLKSGTASVVCLLNNFYPREAKVQWKVDNALQSGNSQESVTEQDSKDSTYSLSSTLTLSKADYEKHKVYACEVTHQGLSSPVTKSFNRGEC

SEQ ID NO: 92 - protein, 214 aa, synthetic construct
DIQLTQSPSFLSASVGDRVTITCRASQGISSYLAWYQQKPGKAPKLLIYAASTLQSGVPSRFSGSGSGTEFTLTISSLQPEDFATYYCQQLNNYPWTFGQGTKVEIKRTVAAPSVFIFPPSDEQLKSGTASVVCLLNNFYPREAKVQWKVDNALQSGNSQESVTEQDSKDSTYSLSSTLTLSKADYEKHKVYACEVTHQGLSSPVTKSFNRGEC

SEQ ID NO: 93 - protein, 583 aa, synthetic construct
QVQLVESGGGVVQPGMSLRLSCAASGFDFSSYGMYWVRQAPGKGQEWVASIRYTGTEKHYADSVKGRFTISRDNSKNTLYLEMNSLRVEDTAVYYCAKNRAIFGVIPDDSDIRGQGTMVTVSSGGGGSQVQLVQSGAEVKKPGASVKVSCKASGYTFAGYYMYWVRQAPGQGLEWMGWINPDSGAPTYAQKFQGRVTMTRDTSISTAYMELSRLRSDDTAVYYCAREKIYYGSGNYYPSFDYWGQGTLVTVSSASTKGPSVFPLAPSSKSTSGGTAALGCLVKDYFPEPVTVSWNSGALTSGVHTFPAVLQSSGLYSLSSVVTVPSSSLGTQTYICNVNHKPSNTKVDKKVEPKSCDKTHTCPPCPAPEAAGAPSVFLFPPKPKDTLMISRTPEVTCVVVDVSHEDPEVKFNWYVDGVEVHNAKTKPREEQYNSTYRVVSVLTVLHQDWLNGKEYKCKVSNKALPAPIEKTISKAKGQPREPQVYTLPPSREEMTKNQVSLTCLVKGFYPSDIAVEWESNGQPENNYKTTPPVLDSDGSFFLYSKLTVDKSRWQQGNVFSCSVMHEALHNHYTQKSLSLSPGK

SEQ ID NO: 94 - protein, 583 aa, synthetic construct
QVQLVESGGGVVQPGMSLRLSCAASGFTFSSYGMYWVRQAPGKGQEWVASIRYTGTEKHYADSVKGRFTISRDNSKNTLYLEMNSLRVEDTAVYYCAKNRALFGVIPDDSDIRGQGTMVTVSSGGGGSQVQLVQSGAEVKKPGASVKVSCKASGYTFAGYYMYWVRQAPGQGLEWMGWINPDSGAPTYAQKFQGRVTMTRDTSISTAYMELSRLRSDDTAVYYCAREKIYYGSGNYYPSFDYWGQGTLVTVSSASTKGPSVFPLAPSSKSTSGGTAALGCLVKDYFPEPVTVSWNSGALTSGVHTFPAVLQSSGLYSLSSVVTVPSSSLGTQTYICNVNHKPSNTKVDKKVEPKSCDKTHTCPPCPAPEAAGAPSVFLFPPKPKDTLMISRTPEVTCVVVDVSHEDPEVKFNWYVDGVEVHNAKTKPREEQYNSTYRVVSVLTVLHQDWLNGKEYKCKVSNKALPAPIEKTISKAKGQPREPQVYTLPPSREEMTKNQVSLTCLVKGFYPSDIAVEWESNGQPENNYKTTPPVLDSDGSFFLYSKLTVDKSRWQQGNVFSCSVMHEALHNHYTQKSLSLSPGK

SEQ ID NO: 95 - protein, 583 aa, synthetic construct
QVQLVESGGGVVQPGMSLRLSCAASGFDFSSYGMYWVRQAPGKGQEWVASIRYTGTEKHYADSVKGRFTISRDNSKNTLYLEMNSLRVEDTAVYYCAKNRAIFGVVPDASDIRGQGTMVTVSSGGGGSQVQLVQSGAEVKKPGASVKVSCKASGYTFAGYYMYWVRQAPGQGLEWMGWINPDSGAPTYAQKFQGRVTMTRDTSISTAYMELSRLRSDDTAVYYCAREKIYYGSGNYYPSFDYWGQGTLVTVSSASTKGPSVFPLAPSSKSTSGGTAALGCLVKDYFPEPVTVSWNSGALTSGVHTFPAVLQSSGLYSLSSVVTVPSSSLGTQTYICNVNHKPSNTKVDKKVEPKSCDKTHTCPPCPAPEAAGAPSVFLFPPKPKDTLMISRTPEVTCVVVDVSHEDPEVKFNWYVDGVEVHNAKTKPREEQYNSTYRVVSVLTVLHQDWLNGKEYKCKVSNKALPAPIEKTISKAKGQPREPQVYTLPPSREEMTKNQVSLTCLVKGFYPSDIAVEWESNGQPENNYKTTPPVLDSDGSFFLYSKLTVDKSRWQQGNVFSCSVMHEALHNHYTQKSLSLSPGK

SEQ ID NO: 96 - protein, 583 aa, synthetic construct
QVQLVESGGGVVQPGMSLRLSCAASGFDFSSYGMYWVRQAPGKGQEWVASIRYTGTEKHYADSVKGRFTISRDNSKNTLYLEMNSLRVEDTAVYYCAKNRALFGVIPDASDIRGQGTMVTVSSGGGGSQVQLVQSGAEVKKPGASVKVSCKASGYTFAGYYMYWVRQAPGQGLEWMGWINPDSGAPTYAQKFQGRVTMTRDTSISTAYMELSRLRSDDTAVYYCAREKIYYGSGNYYPSFDYWGQGTLVTVSSASTKGPSVFPLAPSSKSTSGGTAALGCLVKDYFPEPVTVSWNSGALTSGVHTFPAVLQSSGLYSLSSVVTVPSSSLGTQTYICNVNHKPSNTKVDKKVEPKSCDKTHTCPPCPAPEAAGAPSVFLFPPKPKDTLMISRTPEVTCVVVDVSHEDPEVKFNWYVDGVEVHNAKTKPREEQYNSTYRVVSVLTVLHQDWLNGKEYKCKVSNKALPAPIEKTISKAKGQPREPQVYTLPPSREEMTKNQVSLTCLVKGFYPSDIAVEWESNGQPENNYKTTPPVLDSDGSFFLYSKLTVDKSRWQQGNVFSCSVMHEALHNHYTQKSLSLSPGK

SEQ ID NO: 97 - protein, 583 aa, synthetic construct
QVQLVESGGGVVQPGMSLRLSCAASGFDFSSYGMYWVRQAPGKGQEWVASIRYTGTEKHYADSVKGRFTISRDNSKNTLYLEMNSLRVEDTAVYYCAKNRALFGVIPDDSDIRGQGTMVTVSSGGGGSQVQLVQSGAEVKKPGASVKVSCKASGYTFAGYYMYWVRQAPGQGLEWMGWINPDSGAPTYAQKFQGRVTMTRDTSISTAYMELSRLRSDDTAVYYCAREKIYYGSGNYYPSFDYWGQGTLVTVSSASTKGPSVFPLAPSSKSTSGGTAALGCLVKDYFPEPVTVSWNSGALTSGVHTFPAVLQSSGLYSLSSVVTVPSSSLGTQTYICNVNHKPSNTKVDKKVEPKSCDKTHTCPPCPAPEAAGAPSVFLFPPKPKDTLMISRTPEVTCVVVDVSHEDPEVKFNWYVDGVEVHNAKTKPREEQYNSTYRVVSVLTVLHQDWLNGKEYKCKVSNKALPAPIEKTISKAKGQPREPQVYTLPPSREEMTKNQVSLTCLVKGFYPSDIAVEWESNGQPENNYKTTPPVLDSDGSFFLYSKLTVDKSRWQQGNVFSCSVMHEALHNHYTQKSLSLSPGK

SEQ ID NO: 98 - protein, 581 aa, synthetic construct
QVQLVESGGGVVQPGMSLRLSCAASGFDFSSYGMYWVRQAPGKGQEWVASIRYTGTEKHYADSVKGRFTISRDNSKNTLYLEMNSLRVEDTAVYYCAKNRAIFGVIPDDSDIRGQGTMVTVSSGGSQVQLVQSGAEVKKPGASVKVSCKASGYTFAGYYMYWVRQAPGQGLEWMGWINPDSGAPTYAQKFQGRVTMTRDTSISTAYMELSRLRSDDTAVYYCAREKIYYGSGNYYPSFDYWGQGTLVTVSSASTKGPSVFPLAPSSKSTSGGTAALGCLVKDYFPEPVTVSWNSGALTSGVHTFPAVLQSSGLYSLSSVVTVPSSSLGTQTYICNVNHKPSNTKVDKKVEPKSCDKTHTCPPCPAPEAAGAPSVFLFPPKPKDTLMISRTPEVTCVVVDVSHEDPEVKFNWYVDGVEVHNAKTKPREEQYNSTYRVVSVLTVLHQDWLNGKEYKCKVSNKALPAPIEKTISKAKGQPREPQVYTLPPSREEMTKNQVSLTCLVKGFYPSDIAVEWESNGQPENNYKTTPPVLDSDGSFFLYSKLTVDKSRWQQGNVFSCSVMHEALHNHYTQKSLSLSPGK

SEQ ID NO: 99 - protein, 581 aa, synthetic construct
QVQLVESGGGVVQPGMSLRLSCAASGFDFSSYGMYWVRQAPGKGQEWVASIRYTGTEKHYADSVKGRFTISRDNSKNTLYLEMNSLRVEDTAVYYCAKNRALFGVIPDDSDIRGQGTMVTVSSGGSQVQLVQSGAEVKKPGASVKVSCKASGYTFAGYYMYWVRQAPGQGLEWMGWINPDSGAPTYAQKFQGRVTMTRDTSISTAYMELSRLRSDDTAVYYCAREKIYYGSGNYYPSFDYWGQGTLVTVSSASTKGPSVFPLAPSSKSTSGGTAALGCLVKDYFPEPVTVSWNSGALTSGVHTFPAVLQSSGLYSLSSVVTVPSSSLGTQTYICNVNHKPSNTKVDKKVEPKSCDKTHTCPPCPAPEAAGAPSVFLFPPKPKDTLMISRTPEVTCVVVDVSHEDPEVKFNWYVDGVEVHNAKTKPREEQYNSTYRVVSVLTVLHQDWLNGKEYKCKVSNKALPAPIEKTISKAKGQPREPQVYTLPPSREEMTKNQVSLTCLVKGFYPSDIAVEWESNGQPENNYKTTPPVLDSDGSFFLYSKLTVDKSRWQQGNVFSCSVMHEALHNHYTQKSLSLSPGK

SEQ ID NO: 100 - protein, 4 aa, synthetic construct
GSGS

SEQ ID NO: 101 - protein, 5 aa, synthetic construct
GGGGS

SEQ ID NO: 102 - protein, 7 aa, synthetic construct
GGGGSGS

SEQ ID NO: 103 - protein, 15 aa, synthetic construct
GGGGSGGGGSGGGGS

SEQ ID NO: 104 - protein, 15 aa, synthetic construct
EPKSSDKTHTPPPPP

SEQ ID NO: 105 - protein, 10 aa, synthetic construct
DKTHTCPPCP

SEQ ID NO: 106 - protein, 15 aa, synthetic construct
GGGGGDKTHTCPPCP